European Patent Specification EP 4 056 718 B1, published September 18, 2024. Title: Detection composition of SARS-CoV-2 virus gene and COVID-19 diagnosis method using real-time RT-PCR. Applicant: Industry Academic Cooperation Foundation of Chosun University. The sequence listing filed with the application follows.

SEQUENCE LISTING (10 sequences)

SEQ ID NO: 1 - DNA, 18 bp, Artificial Sequence
  nCoV_RdRp-126F primer sequence
gctggttttgctaaattc

SEQ ID NO: 2 - DNA, 19 bp, Artificial Sequence
  nCoV_RdRp-226R primer sequence
gtgtgtctcttaactacaa

SEQ ID NO: 3 - DNA, 23 bp, Artificial Sequence
  nCoV_RdRp-151P probe sequence
ctaattgttgtcgcttccaagaa

SEQ ID NO: 4 - DNA, 18 bp, Artificial Sequence
  nCoV_3a-63F primer sequence
ggatgctactccttcaga

SEQ ID NO: 5 - DNA, 18 bp, Artificial Sequence
  nCoV_3a-225R primer sequence
cttggagagtgctagttg

SEQ ID NO: 6 - DNA, 24 bp, Artificial Sequence
  nCoV_3a-100P probe sequence
acgataccgatacaagcctcactc

SEQ ID NO: 7 - DNA, 101 bp, Artificial Sequence
  RdRp PCR product sequence
gctggttttgctaaattcctaaaaactaattgttgtcgcttccaagaaaaggacgaagatgacaatttaattgattcttactttgtagttaagagacacac

SEQ ID NO: 8 - DNA, 163 bp, Artificial Sequence
  ORF3a PCR product sequence
ggatgctactccttcagattttgttcgcgctactgcaacgataccgatacaagcctcactccctttcggatggcttattgttggcgttgcacttcttgctgtttttcagagcgcttccaaaatcataaccctcaaaaagagatggcaactagcactctccaag

SEQ ID NO: 9 - DNA, 2795 bp, Artificial Sequence
  SARS-CoV-2 RdRp DNA sequence
tcagctgatgcacaatcgtttttaaacgggtttgcggtgtaagtgcagcccgtcttacaccgtgcggcacaggcactagtactgatgtcgtatacagggcttttgacatctacaatgataaagtagctggttttgctaaattcctaaaaactaattgttgtcgcttccaagaaaaggacgaagatgacaatttaattgattcttactttgtagttaagagacacactttctctaactaccaacatgaagaaacaatttataatttacttaaggattgtccagctgttgctaaacatgacttctttaagtttagaatagacggtgacatggtaccacatatatcacgtcaacgtcttactaaatacacaatggcagacctcgtctatgctttaaggcattttgatgaaggtaattgtgacacattaaaagaaatacttgtcacatacaattgttgtgatgatgattatttcaataaaaaggactggtatgattttgtagaaaacccagatatattacgcgtatacgccaacttaggtgaacgtgtacgccaagctttgttaaaaacagtacaattctgtgatgccatgcgaaatgctggtattgttggtgtactgacattagataatcaagatctcaatggtaactggtatgatttcggtgatttcatacaaaccacgccaggtagtggagttcctgttgtagattcttattattcattgttaatgcctatattaaccttgaccagggctttaactgcagagtcacatgttgacactgacttaacaaagccttacattaagtgggatttgttaaaatatgacttcacggaagagaggttaaaactctttgaccgttattttaaatattgggatcagacataccacccaaattgtgttaactgtttggatgacagatgcattctgcattgtgcaaactttaatgttttattctctacagtgttcccacctacaagttttggaccactagtgagaaaaatatttgttgatggtgttccatttgtagtttcaactggataccacttcagagagctaggtgttgtacataatcaggatgtaaacttacatagctctagacttagttttaaggaattacttgtgtatgctgctgaccctgctatgcacgctgcttctggtaatctattactagataaacgcactacgtgcttttcagtagctgcacttactaacaatgttgcttttcaaactgtcaaacccggtaattttaacaaagacttctatgactttgctgtgtctaagggtttctttaaggaaggaagttctgttgaattaaaacacttcttctttgctcaggatggtaatgctgctatcagcgattatgactactatcgttataatctaccaacaatgtgtgatatcagacaactactatttgtagttgaagttgttgataagtactttgattgttacgatggtggctgtattaatgctaaccaagtcatcgtcaacaacctagacaaatcagctggttttccatttaataaatggggtaaggctagactttattatgattcaatgagttatgaggatcaagatgcacttttcgcatatacaaaacgtaatgtcatccctactataactcaaatgaatcttaagtatgccattagtgcaaagaatagagctcgcaccgtagctggtgtctctatctgtagtactatgaccaatagacagtttcatcaaaaattattgaaatcaatagccgccactagaggagctactgtagtaattggaacaagcaaattctatggtggttggcacaacatgttaaaaactgtttatagtgatgtagaaaaccctcaccttatgggttgggattatcctaaatgtgatagagccatgcctaacatgcttagaattatggcctcacttgttcttgctcgcaaacatacaacgtgttgtagcttgtcacaccgtttctatagattagctaatgagtgtgctcaagtattgagtgaaatggtcatgtgtggcggttcactatatgttaaaccaggtggaacctcatcaggagatgccacaactgcttatgctaatagtgtttttaacatttgtcaagctgtcacggccaatgttaatgcacttttatctactgatggtaacaaaattgccgataagtatgtccgcaatttacaacacagactttatgagtgtctctatagaaatagagatgttgacacagactttgtgaatgagttttacgcatatttgcgtaaacatttctcaatgatgatactctctgacgatgctgttgtgtgtttcaatagcacttatgcatctcaaggtctagtggctagcataaagaactttaagtcagttctttattatcaaaacaatgtttttatgtctgaagcaaaatgttggactgagactgaccttactaaaggacctcatgaattttgctctcaacatacaatgctagttaaacagggtgatgattatgtgtaccttccttacccagatccatcaagaatcctaggggccggctgttttgtagatgatatcgtaaaaacagatggtacacttatgattgaacggttcgtgtctttagctatagatgcttacccacttactaaacatcctaatcaggagtatgctgatgtctttcatttgtacttacaatacataagaaagctacatgatgagttaacaggacacatgttagacatgtattctgttatgcttactaatgataacacttcaaggtattgggaacctgagttttatgaggctatgtacacaccgcatacagtcttacag

SEQ ID NO: 10 - DNA, 828 bp, Artificial Sequence
  SARS-CoV-2 OFR3a DNA sequence
atggatttgtttatgagaatcttcacaattggaactgtaactttgaagcaaggtgaaatcaaggatgctactccttcagattttgttcgcgctactgcaacgataccgatacaagcctcactccctttcggatggcttattgttggcgttgcacttcttgctgtttttcagagcgcttccaaaatcataaccctcaaaaagagatggcaactagcactctccaagggtgttcactttgtttgcaacttgctgttgttgtttgtaacagtttactcacaccttttgctcgttgctgctggccttgaagccccttttctctatctttatgctttagtctacttcttgcagagtataaactttgtaagaataataatgaggctttggctttgctggaaatgccgttccaaaaacccattactttatgatgccaactattttctttgctggcatactaattgttacgactattgtataccttacaatagtgtaacttcttcaattgtcattacttcaggtgatggcacaacaagtcctatttctgaacatgactaccagattggtggttatactgaaaaatgggaatctggagtaaaagactgtgttgtattacacagttacttcacttcagactattaccagctgtactcaactcaattgagtacagacactggtgttgaacatgttaccttcttcatctacaataaaattgttgatgagcctgaagaacatgtccaaattcacacaatcgacggttcatccggagttgttaatccagtaatggaaccaatttatgatgaaccgacgacgactactagcgtgcctttgtaa